European Patent Specification EP 3 137 097 B1, published June 21, 2023. Title: Treatment and prevention of Alzheimer's Disease (AD). Applicant: AFFiRiS AG. The sequence listing filed with the application follows.

SEQUENCE LISTING (2 sequences)

SEQ ID NO: 1 - protein, 7 aa, artificial sequence
  artificially created peptide sequence
SWEFRTC

SEQ ID NO: 2 - protein, 7 aa, artificial sequence
  artificially made peptide
SEFKHGC